European Patent Specification EP 4 134 667 B1, published November 12, 2025. Title: APPARATUS AND METHOD FOR MEASURING ANALYTES USING FET ARRAYS. Applicant: Life Technologies Corporation. The sequence listing filed with the application follows.

SEQUENCE LISTING (7 sequences)

SEQ ID NO: 1 - DNA, 60 bp, Artificial Sequence
  Synthetic Oligonucleotide
gcaagtgcccttaggcttcagttcaaaagtcctaactgggcaaggcacacaggggatagg

SEQ ID NO: 2 - DNA, 60 bp, Artificial Sequence
  Synthetic Oligonucleotide
ccatgtccccttaagccccccccattcccccctgaacccccaaggcacacaggggatagg

SEQ ID NO: 3 - DNA, 60 bp, Artificial Sequence
  Synthetic Oligonucleotide
aagctcaaaaacggtaaaaaaaagccaaaaaactggaaaacaaggcacacaggggatagg

SEQ ID NO: 4 - DNA, 60 bp, Artificial Sequence
  Synthetic Oligonucleotide
ttcgagtttttgccattttttttcggttttttgaccttttcaaggcacacaggggatagg

SEQ ID NO: 5 - DNA, 25 bp, Artificial Sequence
  Synthetic Oligonucleotide
actggtccagcattagccgtacgac

SEQ ID NO: 6 - DNA, 13 bp, Artificial Sequence
  Synthetic Oligonucleotide
gtcgtacggctaa

SEQ ID NO: 7 - DNA, 14 bp, Artificial Sequence
  Synthetic Oligonucleotide
gtcgtacggctaat